European Patent Application EP 4 279 078 A1, published November 22, 2023. Title: Composition for preventing or treating renal disease. Applicant: Industry-Academic Cooperation Foundation, Yonsei University. The sequence listing filed with the application follows.

SEQUENCE LISTING (24 sequences)

SEQ ID NO: 1 - protein, 1093 aa, Homo sapiens [sequence omitted]

SEQ ID NO: 2 - protein, 283 aa, Homo sapiens
MDVLPMCSIFQELQIVHETGYFSALPSLEEYWQQTCLELERYLQSEPCYVSASEIKFDSQEDLWTKIILAREKKEESELKISSSPPEDTLISPSFCYNLETNSLNSDVSSESSDSSEELSPTAKFTSDPIGEVLVSSGKLSSSVTSTPPSSPELSREPSQLWGCVPGELPSPGKVRSGTSGKPGDKGNGDASPDGRRRVHRCHFNGCRKVYTKSSHLKAHQRTHTGEKPYRCSWEGCEWRFARSDELTRHFRKHTGAKPFKCSHCDRCFSRSDHLALHMKRHL

SEQ ID NO: 3 - DNA, 24 bp, Artificial Sequence
  forward primer
ggtgagcctggccttatgtgaata

SEQ ID NO: 4 - DNA, 20 bp, Artificial Sequence
  reverse primer
caccaccatcctgcacctcc

SEQ ID NO: 5 - DNA, 22 bp, Artificial Sequence
  forward primer
tactctttccttcaggcagtga

SEQ ID NO: 6 - DNA, 19 bp, Artificial Sequence
  reverse primer
gatcgaggcaagtgcatgg

SEQ ID NO: 7 - DNA, 22 bp, Artificial Sequence
  forward primer
cacctccacaagaatgaaagcg

SEQ ID NO: 8 - DNA, 19 bp, Artificial Sequence
  reverse primer
ctccgcctcgatgtagtgc

SEQ ID NO: 9 - DNA, 21 bp, Artificial Sequence
  forward primer
aaccttggagtgaaggatcgc

SEQ ID NO: 10 - DNA, 23 bp, Artificial Sequence
  reverse primer
gtaggagagcctattggagatgt

SEQ ID NO: 11 - DNA, 22 bp, Artificial Sequence
  forward primer
ctcaacatttccaatccgaccc

SEQ ID NO: 12 - DNA, 21 bp, Artificial Sequence
  reverse primer
ggcatccttgctcttagtggg

SEQ ID NO: 13 - DNA, 19 bp, Artificial Sequence
  forward primer
gagagccagcctaccatcc

SEQ ID NO: 14 - DNA, 21 bp, Artificial Sequence
  reverse primer
gggtcctcgtgtttgaaggaa

SEQ ID NO: 15 - DNA, 21 bp, Artificial Sequence
  forward primer
aagttcggttttcgctccagg

SEQ ID NO: 16 - DNA, 19 bp, Artificial Sequence
  reverse primer
acaccccggagaggttctg

SEQ ID NO: 17 - DNA, 21 bp, Artificial Sequence
  forward primer
ctcggccattcgtacatggaa

SEQ ID NO: 18 - DNA, 20 bp, Artificial Sequence
  reverse primer
ggatacctctgcaccgtagc

SEQ ID NO: 19 - DNA, 20 bp, Artificial Sequence
  forward primer
gcgtcagggagatggtaaag

SEQ ID NO: 20 - DNA, 20 bp, Artificial Sequence
  reverse primer
catcagggaaacagttgcag

SEQ ID NO: 21 - DNA, 22 bp, Artificial Sequence
  forward primer
cgctaagaatccgctggtgaag

SEQ ID NO: 22 - DNA, 22 bp, Artificial Sequence
  reverse primer
ggatcttgacgaagcagtcgtt

SEQ ID NO: 23 - DNA, 20 bp, Artificial Sequence
  forward primer
cctcgggtcagtttgagctg

SEQ ID NO: 24 - DNA, 22 bp, Artificial Sequence
  reverse primer
ccttgaggcacactttgaagta